European Patent Application EP 4 382 113 A1, published June 12, 2024. Title: Combination Use of Novel Lactobacillus plantarum strain, the strain-derived polysaccharide for preventing or treating tumor. Applicant: Immunobiome INC. The sequence listing filed with the application follows.

SEQUENCE LISTING (4 sequences)

SEQ ID NO: 1 - DNA, 20 bp, synthetic construct
  source 1..20: mol_type = other DNA
agagtttgatcmtggctcag

SEQ ID NO: 2 - DNA, 22 bp, synthetic construct
  source 1..22: mol_type = other DNA
tacggytaccttgttacgactt

SEQ ID NO: 3 - DNA, 1522 bp, Lactobacillus plantarum
  source 1..1522: mol_type = genomic DNA
agcgctgggatgatgctagtgttggagggtttccgcccttcagtgctgcagctaacgcattaagcattccgcctggggagtacggccgcaaggctgaaactcaaaggaattgacgggggcccgcacaagcggtggagcatgtggtttaattcgaagctacgcgaagaaccttaccaggtcttgacatactatgcaaatctaagagattagacgttcccttcggggacatggatacaggtggtgcatggttgtcgtcagctcgtgtcgtgagatgttgggttaagtcccgcaacgagcgcaacccttattatcagttgccagcattaagttgggcactctggtgagactgccggtgacaaaccggaggaaggtggggatgacgtcaaatcatcatgccccttatgacctgggctacacacgtgctacaatggatggtacaacgagttgcgaactcgcgagagtaagctaatctcttaaagccattctcagttcggattgtaggctgcaactcgcctacatgaagtcggaatcgctagtaatcgcggatcagcatgccgcggtgaatacgttcccgggccttgtacacaccgcccgtcacaccatgagagtttgtaacacccaaagtcggtggggtaaccttttaggaaccagccgcctaaggtgggacagatgattagggtgaagtcgtaacagggtaaaaccgtaaagatgttcaacccgccacatctgtcgcgtctccgtcgtagatataagaaagccaaagggcctttcttccatggctgggtgttcatgcaataacatcgaccggttatccacgacacaagaaaggattacgttggtcctggttgtgcgctcaggttttatagtgacagcgggcctatttgtatggtgtaaaccggagtgctaacaatcttctacaagaaacagcctgtacataaatttacggcatatatataccggaacgtggcttggccacgtatgttattaacgcgggctggcaggaacttactaggccgtgccattccggtgtcaaatccgaccgaatccggggactcgtctcgcggaaatgtgtttctttttagagacatggattcttacaaaccgagaccctgtcatgcccgggatgagggtctgccactaacaactttccgaacatgatgggaagaaccccctaacgggcgcccacctggaggaatttgggccggggcaccaccgcccgaggtggggcggaaaaccccctccaggggtcccatcctcaatttttccgggggggacccccctcccccccaaaatgagggaaaacccccgggggggcacccccaaaagaaggagagccccccaccctcactcttcccgcccggcgtgcgggggcgggtttttttttctgtcaaaataaattttgtgttgtttgtgtgttcctcccccccccgccgcgggggcggggttgtacttttttccctctccatcccccccccaccacaaaagaaaaggaggggacgacacccacagtgggtgtgttttt

SEQ ID NO: 4 - DNA, 1554 bp, Lactobacillus plantarum
  source 1..1554: mol_type = genomic DNA
ttgacgggggggtctccaggcggaatgcttaatgcgttagctgcagcactgaagggcggaaaccccccaacacttagcattcatcgtttacggtatggactaccagggtatctaatcctgtttgctacccatactttcgagcctcagcgtcagttacagaccagacagccgccttcgccactggtgttcttccatatatctacgcatttcaccgctacacatggagttccactgtcctcttctgcactcaagtttcccagtttccgatgcacttcttcggttgagccgaaggctttcacatcagacttaaaaaaccgcctgcgctcgctttacgcccaataaatccggacaacgcttgccacctacgtattaccgcggctgctggcacgtagttagccgtggctttctggttaaataccgtcaatacctgaacagttactctcagatatgttcttctttaacaacagagttttacgagccgaaacccttcttcactcacgcggcgttgctccatcagactttcgtccattgtggaagattccctactgctgcctcccgtaggagtttgggccgtgtctcagtcccaatgtggccgattaccctctcaggtcggctacgtatcattgccatggtgagccgttaccccaccatctagctaatacgccgcgggaccatccaaaagtgatagccgaagccatctttcaaactcggaccatgcggtccaagttgttatgcggtattagcatctgtttccaggtgttatcccccgcttctgggcaggtttcccacgtgttactcaccagttcgccactcactcaaatgtaaatcatgatgcaagcaccaatcaataccagagttcgttcgacttgcatgtattaggcacgccgccagcgttcgtcctgacagagagaaaaaaaaaaaaaaaaaagggccggggggatcggggggggggggggggggggtgaggggttgagggggggggggggggggggggggggggggggggggggggggggggggggggggggggggggggggggggggggggggggggggggggggggggggggggggggggggggggggggggggggtgtgtgggggggggggggttgttgtttttgtttggggggggggttgttttttgtgtgtgttttgttgtttgtttgggggtgtgttttgttgtggggtggggtgttgggggggttggggggggggtgttgtttggggggggtgggggggggggtttttttgttgttgtgtggttgtgtgttgtgtggtgggtggggggggtggtgtgtgtgtgggggtggggggtgtttggtggggggggggttgttgtgggggggtggtgtttgttttttgtttttttttgtgtgtggggggggggggtggggggtggtttgtggggtgttgtttgtgtgtggttggtggtggtgtgtgggggggttgggggggggggggttgtcttttttgttggtgttgggtgtttgttggtgttggtgtgtggtggggtggtgtggtgggtgggtgcttgttgtgtgtgtggtgtgt